European Patent Specification EP 3 684 949 B1, published April 17, 2024. Title: IN SITU COMBINATORIAL LABELING OF CELLULAR MOLECULES. Applicant: Seelig, Georg Rosenberg, Alexander B. Roco, Charles. The sequence listing filed with the application follows.

SEQUENCE LISTING (15 sequences)

SEQ ID NO: 1 - DNA, 32 bp, Artificial Sequence
  Reverse transcription primer, top strand
  misc_feature (1)..(1): n is a, c, g, or t
nbaaaaaaaaaaaaaaacgaatgctctggcct

SEQ ID NO: 2 - DNA, 32 bp, Artificial Sequence
  Reverse transcription primer, bottom strand
  misc_feature (32)..(32): n is a, c, g, or t
aggccagagcattcgtttttttttttttttvn

SEQ ID NO: 3 - DNA, 30 bp, Artificial Sequence
  BC_0056_S0-S1
cgaatgctctggccttcggacgatcatggg

SEQ ID NO: 4 - DNA, 38 bp, Artificial Sequence
  Round 1 barcodes
  misc_feature (16)..(23): n is a, c, g, or t
cgcgctgcatacttgnnnnnnnncccatgatcgtccga

SEQ ID NO: 5 - DNA, 30 bp, Artificial Sequence
  BC_0058_S2-S3
caagtatgcagcgcggggaagcacgtggat

SEQ ID NO: 6 - DNA, 38 bp, Artificial Sequence
  Round 2 barcodes
  misc_feature (16)..(23): n is a, c, g, or t
catcggcgtacgactnnnnnnnnatccacgtgcttccc

SEQ ID NO: 7 - DNA, 30 bp, Artificial Sequence
  BC_0060_S4-S5
agtcgtacgccgatgcgaaacatcggccac

SEQ ID NO: 8 - DNA, 55 bp, Artificial Sequence
  Round 3 barcodes
  misc_feature (23)..(40): n is a, c, g, or t
cagacgtgtgctcttccgatctnnnnnnnnnnnnnnnnnngtggccgatgtttcg

SEQ ID NO: 9 - DNA, 191 bp, Artificial Sequence
  Stop ligation oligos, top strand
  misc_feature (1)..(29): n is a, c, g, or t
  misc_feature (76)..(83): n is a, c, g, or t
  misc_feature (114)..(121): n is a, c, g, or t
  misc_feature (152)..(169): n is a, c, g, or t
nnnnnnnnnnnnnnnnnnnnnnnnnnnnnbaaaaaaaaaaaaaaacgaatgctctggccttcggacgatcatgggnnnnnnnncaagtatgcagcgcggggaagcacgtggatnnnnnnnnagtcgtacgccgatgcgaaacatcggccacnnnnnnnnnnnnnnnnnnagatcggaagagcacacgtctg

SEQ ID NO: 10 - DNA, 191 bp, Artificial Sequence
  Stop ligation oligos, bottom strand
  misc_feature (23)..(40): n is a, c, g, or t
  misc_feature (71)..(78): n is a, c, g, or t
  misc_feature (109)..(116): n is a, c, g, or t
  misc_feature (163)..(191): n is a, c, g, or t
cagacgtgtgctcttccgatctnnnnnnnnnnnnnnnnnngtggccgatgtttcgcatcggcgtacgactnnnnnnnnatccacgtgcttccccgcgctgcatacttgnnnnnnnncccatgatcgtccgaaggccagagcattcgtttttttttttttttvnnnnnnnnnnnnnnnnnnnnnnnnnnnnn

SEQ ID NO: 11 - DNA, 214 bp, Artificial Sequence
  3' adapter ligation
  misc_feature (24)..(52): n is a, c, g, or t
  misc_feature (99)..(106): n is a, c, g, or t
  misc_feature (137)..(144): n is a, c, g, or t
  misc_feature (175)..(192): n is a, c, g, or t
ggatgtgctgcgagaaggctagannnnnnnnnnnnnnnnnnnnnnnnnnnnnvtttttttttttttttgcttacgagaccggaagcctgctagtacccnnnnnnnngttcatacgtcgcgccccttcgtgcacctannnnnnnntcagcatgcggctacgctttgtagccggtgnnnnnnnnnnnnnnnnnntctagccttctcgtgtgcagac

SEQ ID NO: 12 - DNA, 214 bp, Artificial Sequence
  PCR #1, top strand
  misc_feature (24)..(52): n is a, c, g, or t
  misc_feature (99)..(106): n is a, c, g, or t
  misc_feature (137)..(144): n is a, c, g, or t
  misc_feature (175)..(192): n is a, c, g, or t
cctacacgacgctcttccgatctnnnnnnnnnnnnnnnnnnnnnnnnnnnnnbaaaaaaaaaaaaaaacgaatgctctggccttcggacgatcatgggnnnnnnnncaagtatgcagcgcggggaagcacgtggatnnnnnnnnagtcgtacgccgatgcgaaacatcggccacnnnnnnnnnnnnnnnnnnagatcggaagagcacacgtctg

SEQ ID NO: 13 - DNA, 214 bp, Artificial Sequence
  PCR #1, bottom strand
  misc_feature (23)..(40): n is a, c, g, or t
  misc_feature (71)..(78): n is a, c, g, or t
  misc_feature (109)..(116): n is a, c, g, or t
  misc_feature (163)..(191): n is a, c, g, or t
cagacgtgtgctcttccgatctnnnnnnnnnnnnnnnnnngtggccgatgtttcgcatcggcgtacgactnnnnnnnnatccacgtgcttccccgcgctgcatacttgnnnnnnnncccatgatcgtccgaaggccagagcattcgtttttttttttttttvnnnnnnnnnnnnnnnnnnnnnnnnnnnnnagatcggaagagcgtcgtgtagg

SEQ ID NO: 14 - DNA, 292 bp, Artificial Sequence
  PCR #1, top strand
  misc_feature (59)..(88): n is a, c, g, or t
  misc_feature (135)..(142): n is a, c, g, or t
  misc_feature (173)..(180): n is a, c, g, or t
  misc_feature (211)..(228): n is a, c, g, or t
aatgatacggcgaccaccgagatctacactctttccctacacgacgctcttccgatctnnnnnnnnnnnnnnnnnnnnnnnnnnnnnnbaaaaaaaaaaaaaaacgaatgctctggccttcggacgatcatgggnnnnnnnncaagtatgcagcgcggggaagcacgtggatnnnnnnnnagtcgtacgccgatgcgaaacatcggccacnnnnnnnnnnnnnnnnnnagatcggaagagcacacgtctgaactccagtcacgatctgatctcgtatgccgtcttctgcttg

SEQ ID NO: 15 - DNA, 292 bp, Artificial Sequence
  PCR #2, bottom strand
  misc_feature (65)..(82): n is a, c, g, or t
  misc_feature (113)..(120): n is a, c, g, or t
  misc_feature (151)..(158): n is a, c, g, or t
  misc_feature (205)..(234): n is a, c, g, or t
caagcagaagacggcatacgagatcagatcgtgactggagttcagacgtgtgctcttccgatctnnnnnnnnnnnnnnnnnngtggccgatgtttcgcatcggcgtacgactnnnnnnnnatccacgtgcttccccgcgctgcatacttgnnnnnnnncccatgatcgtccgaaggccagagcattcgtttttttttttttttvnnnnnnnnnnnnnnnnnnnnnnnnnnnnnnagatcggaagagcgtcgtgtagggaaagagtgtagatctcggtggtcgccgtatcatt